European Patent Specification EP 3 679 159 B1, published June 17, 2026. Title: DIAGNOSTIC AND THERAPEUTIC METHODS FOR CANCER. Applicant: Genentech, Inc. The sequence listing filed with the application follows.

SEQUENCE LISTING (6 sequences)

SEQ ID NO: 1 - DNA, 65 bp, Artificial Sequence
  Synthetic Construct
gatcccccttacgctgagtacttcgattcaagagatcgaagtactcagcgtaagttttttggaaa

SEQ ID NO: 2 - DNA, 65 bp, Artificial Sequence
  Synthetic Construct
agcttttccaaaaaacttacgctgagtacttcgatctcttgaatcgaagtactcagcgtaagggg

SEQ ID NO: 3 - DNA, 65 bp, Artificial Sequence
  Synthetic Construct
gatccccgacatgaaatccaacaatattcaagagatattgttggatttcatgtcttttttggaaa

SEQ ID NO: 4 - DNA, 65 bp, Artificial Sequence
  Synthetic Construct
agcttttccaaaaaagacatgaaatccaacaatatctcttgaatattgttggatttcatgtcggg

SEQ ID NO: 5 - DNA, 21 bp, Artificial Sequence
  Synthetic Construct
tcctgcgtctagaggttccca

SEQ ID NO: 6 - DNA, 21 bp, Artificial Sequence
  Synthetic Construct
taggagtagacatccgactgg